European Patent Specification EP 3 381 930 B1, published April 16, 2025. Title: SOLUBLE FORMS OF HENDRA AND NIPAH VIRUS G GLYCOPROTEIN. Applicant: THE HENRY M. JACKSON FOUNDATION FOR THE ADVANCEMENT OF MILITARY MEDICINE, INC. Application PCT/US05/24022. The sequence listing filed with the application follows.

SEQUENCE LISTING (15 sequences)

SEQ ID NO: 1 - DNA, 40 bp, Artificial Sequence
  Description of Artificial Sequence: Synthetic oligonucleotide
gtcgaccaccatgcaaaattacaccagaacgactgataat

SEQ ID NO: 2 - DNA, 45 bp, Artificial Sequence
  Description of Artificial Sequence: Synthetic oligonucleotide
gtttaaacgtcgaccaatcaactctctgaacattgggcaggtatc

SEQ ID NO: 3 - DNA, 39 bp, Artificial Sequence
  Description of Artificial Sequence: Synthetic oligonucleotide
ctcgagcaccatgcaaaattacacaagatcaacagacaa

SEQ ID NO: 4 - DNA, 45 bp, Artificial Sequence
  Description of Artificial Sequence: Synthetic oligonucleotide
ctcgagtagcagccggatcaagcttatgtacattgctctggtatc

SEQ ID NO: 5 - DNA, 46 bp, Artificial Sequence
  Description of Artificial Sequence: Synthetic oligonucleotide
caaggagaccgctgctgctaagttcgaacgccagcacatggattct

SEQ ID NO: 6 - DNA, 54 bp, Artificial Sequence
  Description of Artificial Sequence: Synthetic oligonucleotide
aattagaatccatgtgctggcgttcgaacttagcagcagcggtctccttggtac

SEQ ID NO: 7 - DNA, 31 bp, Artificial Sequence
  Description of Artificial Sequence: Synthetic oligonucleotide
cgaacaaaagctcatctcagaagaggatctg

SEQ ID NO: 8 - DNA, 39 bp, Artificial Sequence
  Description of Artificial Sequence: Synthetic oligonucleotide
aattcagatcctcttctgagatgagcttttgttcggtac

SEQ ID NO: 9 - DNA, 34 bp, Artificial Sequence
  Description of Artificial Sequence: Synthetic oligonucleotide
tcgacccaccatggagacagacacactcctgcta

SEQ ID NO: 10 - protein, 21 aa, Artificial Sequence
  Description of Artificial Sequence: Synthetic peptide
METDTLLLWVLLLWVPGSTGD

SEQ ID NO: 11 - protein, 15 aa, Artificial Sequence
  Description of Artificial Sequence: Synthetic peptide
AAQPARRARRTKLGT

SEQ ID NO: 12 - protein, 15 aa, Artificial Sequence
  Description of Artificial Sequence: Synthetic peptide
KETAAAKFERQHMDS

SEQ ID NO: 13 - protein, 10 aa, Artificial Sequence
  Description of Artificial Sequence: Synthetic peptide
EQKLISEEDL

SEQ ID NO: 14 - protein, 15 aa, Artificial Sequence
  Description of Artificial Sequence: Synthetic peptide
NSADIQHSGGRSTTM

SEQ ID NO: 15 - protein, 421 aa, Hendra virus
GLPNQICLQKTTSTILKPRLISYTLPINREGVCITDPLLAVDNGFFAYSHLEKIGSCTRGIAKQRIIGVGEVLDRGDKVPSMFMTNVWTPPNPSTIHHCSSTYHEDFYYTLCAVSHVGDPILNSTSWTESLSLIRLAVRPKSDSGDYNQKYIAITKVERGKYDKVMPYGPSGIKQGDTLYFPAVGFLPRTEFQYNDSNCPIIHCKYSKAENCRLSMGVNSKSHYILRSGLLKYNLSLGGDIILQFIEIADNRLTIGSPSKIYNSLGQPVFYQASYSWDTMIKLGDVDTVDPLRVQWRNNSVISRPGQSQCPRFNVCPEVCWEGTYNDAFLIDRLNWVSAGVYLNSNQTAENPVFAVFKDNEILYQVPLAEDDTNAQKTITDCFLLENVIWCISLVEIYDTGDSVIRPKLFAVKIPAQCSES